European Patent Specification EP 3 613 278 B1, published July 2, 2025. Title: PLANT REGULATORY ELEMENTS AND USES THEREOF. Applicant: Monsanto Technology LLC. The sequence listing filed with the application follows.

SEQUENCE LISTING (44 sequences)

SEQ ID NO: 1 - DNA, 1500 bp, Coix lacryma-jobi
gttgacgtcggaagtgatccgaatcaaacaccaacagggctagaacgcccggagagcgaggttgcagttcaacctgctgagacagcagggaccctggctaaaccgacgaaaaccgatctagagaccggtttagatcgatctagggtttcgggctcctgtgttgataactctagaactcctcccgggaagacccgtaggggagaagcacgtagaggttgtcctaggaccagcaaggccgcctagaacgccgtcaagtctcgtcgggagacgcgccgaacagcaaggtagaaggaaaaaggggtaaaagggtagtagattgattttgatcgattagggtcggatgcctcaatcggccatgatcctctcatatatatagagggggctggtcttatcccaataggaaacatctccggatacgatctccaagcttcctatccggactctatcaacatatagaattcaatccggacgtgacaaggtaaccctgatttcgccgatccttggatcgaccagatcggtctaatgggctttatcagcccatactgatcaacaaatcgtccttacaagagaaggatccacatacttagcgtcggactcagcaatcatcacaaccataaggcctccaaccagggccacctggtcggacataacatgagtgatcggaaacccaaaatgatcaggcccattcaacttagaacatctgatctctcaaaagacaaattcgaccttaatattacaggccgaatacttcttctaaattcatttttatctgtgacacttttgagtgtcaacagtatgcttttctttgcaaatattcccttttttatttctacccattagttactttggcccttccatttcattgtatgtaaaagtggatactaaagctaacgcaacaagaacaaaaataaatagatccggggtatgacgtccccacggatattttactaaaatatcttctcatcagatctagaaaatcctcgggccctatccatatagggtggtatcacatccatatacttatagtaggacagatgaggagatttttttaccctcaattctaaaattcatcactttaattaaaggaatttaactcaggaccagagcggtgtcgcgagagccatatatgtaaccaaaatacctattagtttagggcagcagcaaataaaccattattcctttgtccccttattccgtctccagctagctaaaagctgtacatatgattaatcatcgacatcgtgcatgcaatttgcaggaaagtgcaaggagcagccaggtgtatacacgtctgtagggttcgcgtcacatcgatcacatggatatgcatgcatccaaaacacacgtacgtacacttgctggtgcatgccttatgaaatggaatactacacgcatgtccacaagttaagcacgcacaggcacacacacagagagacacagttgctcgctcaatgcaattggctggtctataaataccaccgaagagaaccatcctaaaga

SEQ ID NO: 2 - DNA, 86 bp, Coix lacryma-jobi
acacaccggtagcgattcgatccttcagaagagctactgctagctagctagagctatcatctgatcggtagcagcaatataattca

SEQ ID NO: 3 - DNA, 594 bp, Digitaria sanguinalis (L.) Scop.
accaacaagcatcatgacaatggcagcaaagcattcgtcagagacgaccaacaagcatcacgacactggcggcaaagcatatcaaaacaatgtaatgagatacaatattgtttcataaagaagcctacctgcatgatcctttctaacaaactcaaaatgataagggccatgctctgttcggtgacaaccttcaaggcatctactttgccagaatttagctttgttattaccagcttgttattagttcttactatccagtctcgaacaacttgggcgccctttgtctcatcatacctctacatactgccctccctgatcaacacaacattcttcaacccaatcccttggcatttgcgcatgttacaaggtgcaaaacagccagcccatattgcaagttactaaactaaactatggtccaaatgcagcaatcttgatcgctagtactgtccggcattatatctgaaacaagtccagatcacccatctcatcacagtcacatgcattcgcgttcacggaaaccgttaacacaccaccaactagtcagcattgcaccaatcttcctccctataaatgcagcaacaatcgagcgacacc

SEQ ID NO: 4 - DNA, 88 bp, Digitaria sanguinalis (L.) Scop.
aacaccacgaaccatcacaggcacttatagcaacaatcaagttatttctgccttgtgcactcgtggtcgagtagtaatacatagcaaa

SEQ ID NO: 5 - DNA, 1500 bp, Digitaria sanguinalis (L.) Scop.
ttgccggcctgtgtgatgttgcgcccccaccaacctttgattttgcctgctgccttgtcagccaacggttggtagtccaccctcttcaaacgtcgcaccgaagttctgtcgactcccagagaaaatattgtatgtaacatatactattactactacagctgaacacgtaacaatatgatcttatttgtgtatgccgaaagcaccgtgctaaagaccacctatcgccctggttgggatcgaggccttgctgctcagccggttgcatcagacgtgtgcgtgcatcgcatgactggcatgtgagttgtggttcataaataatgtctaacaatattaaggtaattcctagtatgcgttgggatcattttttgatgttggatcttgcggcaggtctcacccatgcatgacggattgagaacaagggagactggaccagcatgtaaaagataatgatgaaggcgagccatgttgacggtgtaccgggacaggcagacgcgggccaacatcgaagagggagatagcgtgcgtgctaatgtttttgtggctcgcatgttcaatgactcatacagatttcggtagcttgctaaaatcattcagcttgtcggcaagcatgggccaaacaatctagcaacaatccatgtttgccatcgatgcaataggaagtaatagaatccacttagcttctagatctcacctggatcctccttttatttatatgcatatattttgtggtagtggaggcacacatctttatgtttcatggataatattttgttatatgtatatctgtccaaataaataacgtacgtgtccttcaatcttagactccagttagattgatcaatgtagtggtcttccatattccttttgtgttttgtgtgccatgtctcaagcatgcatgtggaatgaaaagctggaagcttggcatcaattgcctaaggagccataccataaattaaaccatttgctgatatggccacaatttttttaacaagctatgccatagtcattcatgtgccacggttgttgaatcgcctcaattacgtgtggaacatgatggtgttttaaacaacacttggtgatttctattctggcctactcttgcatctaggatcgtgttgttagccatgtgcacatatttagctagctagtagcaaaggcatgagtgagttgctgatgggtttacaaataccagcataagtattcattaatttgaagtgaagcacgttcatgaacatatgagaaaacttacattataatttgcttggtcagatgaaaacctagctgattccttggcgacgacaacatccctccttgttccatactttcttaataattatttttctcccaaaaagtccatcgcgctagcatcaatgaagaaatataagaaaaatcctcatatccacatagtaaatagagcattatgcggtccatgtaggaatcaccttgggagcacctgcttgctcaatcacactataaataccacccatacactgcttcaag

SEQ ID NO: 6 - DNA, 104 bp, Digitaria sanguinalis (L.) Scop.
agaaccatcacagacatacgctacacgcaccctgtacgaacaaccaacctagctagctacctactgaaaacacacataagcttgctaggcagcatatcatagca

SEQ ID NO: 7 - DNA, 1407 bp, Digitaria sanguinalis (L.) Scop.
atcttcaagatgtcgtaatcgatttcttgagtcaaatattttgttttcatattatttagggagtttttcatatggacaatacataaaaatatatatgcagtgcaagttatttttgtttacttattcaatttatccgttcaatcccctaaacaaaattttaccctaaactattttatttggtccaatctacaccctaattatatttctctttttatttctctgtgtctgagttaaattttgacttcaaattttatgaatagatgcaaaacatgatgctttatgctaaaaatttttactaagaaattttctttgttatgttcataggtcaagaatatttaatatgaaattgatcttacatatataaaactgtacaaaaagtaatcatgaaaaaaattaatatatttgttctaacatagagcattatgtataagtcaactgacaaaatttgaaattaaaactcagcttgcatgtgaagaaacaaaaaaagagaaatctaattaggggtagattggaccaaataaaatagtttaagggggggtaaaatgagccaaattttgttcaaggggttaagtggatcaagtaaatagatgaggggggtaaaatggacttttttcaacaattaacctcatctatagaagggtaggtgcatctcagttcgaaaaataagatgcatttggatcttgaaaaatcaatttcccctcacacccccaaatggaaattgtcgtcactactcagataactaatgaaagtagactcttattgtgatgatccaaaaggtctctgtgattggaatttcgtccacactattttcacaacatcgtaatgagatataatattgttccaccagaaagcctacctgcatggtcatttctaataaccaactcaaaaaatggtaaatgacatgctcttttagtgaaaaactttaaggaacctagcttgccaaaatttatctttgtcattaacaactcagtttcaaccatccagtctcaaacaacttcacttttttttttgcgggtaaaacaacttcactttacatgtggccaaattgaacacaacagtcacgtcccattgaggtacctagcaacttgggcatcctttgtctcgtacctctacatatttttgtccctgatcaacacaacattcttaaacccatttccttggcatttgcccatgttacaaggcgcaaaacaaccaacccatatggcaatttactaaactaaactatgctgatccaatgcagcaatcttgatcgctagtactgtccagcattacatctgaaacaagtccagatcacccatctcatcacagtcacatgcatccatggtcacgggaaccgttaacacacaccaccaactaatcggcattgctccaatcctcctataaatacagcaacgatcaggcgagaca

SEQ ID NO: 8 - DNA, 90 bp, Digitaria sanguinalis (L.) Scop.
atacccaatcacacacagtgttagcacttagcaaccgaggtatttctgcgagctttgtgcccttcttgtggtcgagtaattagtagcaaa

SEQ ID NO: 9 - DNA, 583 bp, Miscanthus sinensis f. gracillimus
tctgctagatgcaacgagctggaagccaggcctgggacaactcgttgatgggcgtggggttcatcaaacagagattagcttatcccattttatgtagatgtgccatgtatgcatatgttttggaataatggtgactcgtgaggaagcccgtgcacatgttttggaatgatttctgccaccgatcgcagaattcaaaataaggcgagcacatcagtgtttcgttaaaataataaacggtagattgaaataatgattccagctagcactatatattgtatttctacgttaataattttatatattgcataagggtcctcctaattcatgcatcactagtagctagcacgttgagtgtatttggcatggtttctcaacttgcttcccctgtatcctgatcgatctctccttcataactggcacatcccaggacaaccaggcaacgctcaaatcacacatgcgttgctgattatccacgctgcatgatgcacgaagccaatcactaaagcatcaccttccacaccatcgttcagctataaaaaccctgccaaactgcgtgagaggaccatcccaaagcacaagagca

SEQ ID NO: 10 - DNA, 61 bp, Miscanthus sinensis f. gracillimus
cgaagtgcagcactaaagcaccacttcctgctcacaccgttgtagtaataatccatcacca

SEQ ID NO: 11 - DNA, 1500 bp, Miscanthus sinensis f. gracillimus
ttgtgagacaaaaacactgttgcggctgggaataagccggctgataagttcaagcgaacaggctgtactttagtgcttctatttgaaccattggttctcactctggctatgcattgttgcattctcactctggcttataattttttcttgcctagtaatagtttttgaaataatgggagcaaccacttcagttataatataatgtttgtatgttataatgggagcaatcactctggttaattgttgcctgtttataccatgcaggctgcattatattaattgcttagttccttcttgtttgtatgtgactatgagatttttgtgacctctacaggaagtgaagggaagaggattcctgctggtttcaacagacatagcaagcaaagggtttgcttctctgattgtgtatctagatcacagtagtgtgaatgtgcaccaagcaaaacttaaattaggtgctctatccatgtacattaagcctagctgtatcaaaaaaaattcggtgttatctgcgtaatattggatgtatatataagattctggcattggaatttatattttttttttgtttttaattcattatcacagacgcgtgttggtcgtgcgcgtctgtcataaggtgtcgtcacagacgcgttttgactatacgcgtctgtgatagggttactacagacgcgtctttactccaccagtctgtcttataacctaatcgcagacgcgtgtttgcataacgcagacgcttattggtaacacgcgtctgtagaagaaacttattacagacacgttattaagcgcgtctgtgatgtgtcttaacacgcgtctgtaatgtggatttattacatagtgatcggcccatatgaacgaatgatcgatctaggcccaaagttagtgtatgaaatgttcatttacgtttcaatgcggtttctcaaaaaaaaacgttccaatgctaaacaaaaacataggaattatatagttttgctgtggcttagtaacttcgtccaatcgtgctagtttaatttgtatatacctgtaccatgctattcctctggccttggttcttgcgcatccattattaatgaccacgccacgccacgcattcattcttaatcaccagttgcttgacatccaatgtcctctccactacttgcgcacaccgtctgatactccaagatcccaagctaagataacacccagtgatcatatatataaaaacaaacgccagtgcgagcctggccatttgcggagccaaccgaagccgtgcacaaaatattcgataccgtatcagggaaaacactagttatacgaggtaggcaataatccatgtttcaaaaaaaacaggtaggcaataatccagatcggactcttcctaaccgggttcacatgcatatatgaatatgatggccgggttcacatgaacgctagatatcgtgcctagtagtgcaccgatttcttaatcccgaggctggactataagtacccctggtaacaccgtgatcaaag

SEQ ID NO: 12 - DNA, 98 bp, Miscanthus sinensis f. gracillimus
catcgcaaacaagctgctaatcacttctcaagagctctctaactacattaattagctagagtgatccgcgaggtagctggcttgtgatcgagcaatac

SEQ ID NO: 13 - DNA, 740 bp, Tripsacum dactyloides
aaatggatgaaacaacttggaccaatcagagatggccacgtcagctcccgatcgtcgtaaccgaccaaacccgatcgataacggtttaggctccaatacaccgtcggtaccacccggtcgctatcatctgcccccgtcccaacgctattggtatcgtccgcccctatatcggtcggtagcccagtccaccgtcggggccaatcgtcccctgctgcgtccgctcgtgtcggtaccgatcgccaaaaacgccacgtcaacggcactgcggtaccgaccgccgctggcaccggccttagcgggccacacgaccgatcgctgttgtacggacgtagaggtgaatcatgcgattgaattttcgctagaggaaagttatcatcttattatctccaaccctccttcctacggctggatccgacgaaaatttaccctggacggtgccagtaacaattgcaggtctcactcacgtgctaaatccagcaatcaaacacgaaggaatatacgtgatctggccagaacatgcaagagaataatacagtagtgttagagtacgaaacctacacgattcaacgaattaatcaatgggttcacgttcacgggtatgctcgcgcacgtccaaaatccaacgacatttttataagcggcatgatccagacgggccagctcgagcaccacatggcgtggctccatctcgcatcccccatcaccgctataaataccattggccatgcacacccgcactc

SEQ ID NO: 14 - DNA, 91 bp, Tripsacum dactyloides
ccacacagcacaagcagcagcagcagcagcagctcgatcgaactagcttagctactacgtgcgcgtgcaacaagcagctcgatcgatcgcc

SEQ ID NO: 15 - DNA, 903 bp, Tripsacum dactyloides
actataattttcatagagaccatttctccctccataccatttaaaaaattcaaacaaaaaatatctataagtggccctaggttaagaaaagtgccagtggaaatgcatctttattgacggttttcttgtatctattgccagtaaaaatcatatatttacattggcgattctttgaagcataccgtcatgacaaatctgatttctattgacagaatgcttaagagaatcgctattggtcatttagttgcagcatttaattggtatgttagtctatgaaatagggaagtggaattttgtattgagagatattgtttcattcttagttttacgacacctttgatgatgtagcagcgctggaaagagtgttatgaaattcctattgagaatagccttacaggtcaacagcatacttttaaaattaaaccagagatataccaaacttcagtttctacgatataatatttttctacctcataagttataatcagtggtacctccttttttttatatccctttattaaggacggtagagaacgtcctctactcgtatgttgtacaccaccggtaacgcaattaagtaaaacatgcatgtcaagtagtaagtatataagttggcaactcaccagatggcaggagtcctgacccatcaccggctagctatagctcttgttacgtgaattcagcatgattgctcaacttgcttctgtatttccacatgggggagaattgtcatatctccccctaacaactggcgcgtccagagacaaccatgcaatgaccaaaccgatcgaatcacacatgctttgcagcattcatgtaccaatgctgccaagcacgaaagcatctccctctccgctccatccatcgtcagctataaaaaccatgccaagcaccctgtgaaaa

SEQ ID NO: 16 - DNA, 69 bp, Tripsacum dactyloides
gcatcccaaagcacacaagagcacgcagtgcagcactcaagcacttcctgctcactgcacaccgtacca

SEQ ID NO: 17 - DNA, 1500 bp, Tripsacum dactyloides
aaaaggcacttttctcaagaaacagagttagagatcaaaccaaagtgctagaaacattgtaataggtatgtgcaacatatttaaaggttcaaacctcacagttttaccctttttcacaaagttgcacttcctggcctcgtttaagcttatttggacttagaatcttcaaattgtgctcgattgaacctttactcatatacttagcaaacaagttagtccaagatgttgtgttggacattcaatcaccaaaacttatggaaatggcttaattgcccatttccctttcatggtacaatttgtttcacagatttaagcagaagctatatcaaacacggcgcttctacaacagcttatcagtttagttgcttctcagaatgaaaggtaataaacataagctgctttttactagatccttagataagttgcttttttaacaagcagctctgccaagcagggccatagtgccatgttgtaggctggtcgctttcccgagccatatgaaggtcgtcggtccatgtggctgaaattaaagttgataggcccatcggaacaaatggtcaattagaggcccaaaatttgtgagtcaaattttcatttacacttccacgctagtaaacgaaaacatatatagtacctatatatcgattttttttttctggtgtcttagaaacttcgtccaataatcatgctagtttaatttgtatacctgcacaaagctattcctctggccttggttctttgcgcgtccatgcttgtttatggatgattgcagccacgccacgcattcattctcaatcaccatttgcttgacatctaatgtcctctgcaccacttgcgcacgctacacaccgtctgatacgccaggatcccaagctaaaataacacccaatgatcatgtgaaaacaagtgacagtgcgagccagcccatgcagcgatcttggccatttgcggagccaaccgaagccgtgcacaaaatattcgataccgtataaggggaaacactagttatacgaggtaggcaaatataatcctcttcctaaccggcggccgggttcacatgcatatatgatggccgccagccgggttcacatgatgaacgctatggtgcctagtgcacgatttattaatctcccgaggctgtactataaatacatcggtaatactgtgatcaaagcatcgcaaagaagatctctaagactgtctccagcaacgtcctctatatctatcctctatatctgtcctttacagtctcctctaaaagattccatcctctatatctccttcctctccaacaacggcctctaaatcacgtcctctatacgcaaatacctatattagagacatttttaattttttaatttttgtacatacgtatttgtcatactctcaaatgtattgtacatattttagttttgctaaaccggttgtttaaagtattcaaatggatagaggagaggagagagaaactctatatatagaggatccagcagcgtcctctaa

SEQ ID NO: 18 - DNA, 172 bp, Tripsacum dactyloides
atttagaggaccgtttagaggacgctgctggagggagtagaggacgacagcgttctctaaaatttagagtacaggatactttagaggacctgctggaggcagtctaacaactgcatttggctagagagagtgatcgcgaggtagctagctggcttgtgatcgatcgagcaaa

SEQ ID NO: 19 - DNA, 645 bp, Saccharum officinarum
caaattaaagttgataggcccatcggaagaaatgatcaatgtaaggcccaaaatttgtgtctgaaatgttcgtttacattttcaagctaaataaaaacataggaattatatagttttgctggtggcttagaaacttcgtccaaaatattaaaaaaaaagaaaagaaacttcgtccaaaatggtgcttagtttaatttgtatacctgcaccatgctattcctctggccttgttcttttgcgcatctatccatgcctatggatgatcgcagccacgccacgcaattcattcttaatcaccatttgcttgacatccaatgtcctctacaccaccacttgcgcaccctacacaccggccatttgatacgccaagatcccaagctgaaataacacccaatgatcatatgaaaacaagcgtgagtgcgagcctgcccatgcagcgatcttggccatttgcggagccaaccgaagcccgtgcacaaaatattcgagaccgtataagggaaaacactagttatacgcaatgtccacaataatccagatcgactcttcctaaccgggttcacatgaacgctgttgtgcctagtgcaccgatttcttaaatcccaaggctcgactataaatacccctggtatttgcaccgtgatc

SEQ ID NO: 20 - DNA, 86 bp, Saccharum officinarum
aaagcatcgcaaacaagctaaagagctctctaactacattgattagagtgatctgcgctagaaggaggctagcttgtgatcgagca

SEQ ID NO: 21 - DNA, 1563 bp, Setaria italica
agacccagcaacctaccgagggggtacccgaggtagtgttttgtggtggggctcgtcgaagatcaggaacttgaaggtgaactcgaacacacgatttagacaagttcgggctgcttatgccgcataataccccatgtcatgtgtgttggttggattgtattgattgatcagatatttggagggggccctgcctcgccttatattgcccattgccggaggcagggctacaggtcggttgttgtacaagagtactagtcggttttgaccagcgagtcctactctaattgctacaagtagtttcctaatccttgactagtccttgtccgccacgtagaccacgacgtcttgcacctagtctctgtgtttgatacatcttggtgtacagtccgatattgtaggactatccaagcttcccagtaggcccatagatgtatggccgacaactggataatgtaactctgggtcagtactatccttatctatatagacacaaacaacgtactatagcagaagtttaagctcgtaacccaccaatatttggtggcatagaccacgtattgctgatatagtgctcgtaacccaccaatatttcgtggcatagagatctcttaggcaataaattagcagtacgaaacaatctatgtccacgtgttgctaatacaatgttctaaaccttacagcctactggacagttctctagccatgatacatgtgcatgtccgaacaaatatttatgggtacccgaaaggttaattttttgtagtatttatgagggggaggggggcgttgacgaaaaaaataacttagctaagcgtaattggcttaaaaacatacaatgttgttccagcatcaagcctacgtgatcatttcacaaaaccaactcaaaagataggtgtcatgttccttttagtgcaaaacttaaggacacctaccttgcaaaacttagctttgttacccagaatgaaccgctaagctcgaggagctctgaacttacatgaccaaatatattaaacacaaaagtcatgcatgattttctttaataagtatcgagcaatatggttcgggtgtctttcgtctcatacctctattgtcctccgtgatcaacaagggtggatccgggtggtgcaagggggctcaagcccccctacctctcccaaaggagaaagaagggagaagaaagtgaaggaagaagaaaccccctatattctaatgctacctccgccactgctgatcaacacaacattcttaaaaccatttccttggcatttgcgcatgttacaaggtacaaaagagccagcccatatgccaagttactaaactaaactatgatccaccatggagcgagaacaaacgtcaacaggcatcaaccaatgcagcaatcttgatcgctagtactgtccggcattatatctgaaacaaatccagatcacccatctcatcacagtcacatgcattcatggtcacgggaaccgttagcaaaccaccaactaatcagcattgcaacactcttcctcctataaatgcagcgagcgggggacaccataaaccatcacaggcacttag

SEQ ID NO: 22 - DNA, 67 bp, Setaria italica
cgatcaagttaattttgtttctgctttgtgcgcctgtgttccagtaattactttccgtgtagcaaaa

SEQ ID NO: 23 - DNA, 1528 bp, Oryza sativa
ggaagctaactagtcacggcgaatacatgacgacatcggcctacaacgcacaacttcttggcataaaagcttcaatttcaatgcccctatctggaagccctaggcgccgcgcaaatgtaaaacattcgcttcgcttggcttgttatccaaaatagagtatggacctccgacagattggcaacccgtgggtaatcgaaaatggctccatctgcccctttgtcgaaggaatcaggaaacggccctcacctcctggcggagtgtagatatgtgaaagaatctaggcgacacttgcagactggacaacatgtgaacaaataagaccaacgttatggcaacaagcctcgacgctactcaagtggtgggaggccaccgcatgttccaacgaagcgccaaagaaagccttgcagactctaatgctattagtcgcctaggatatttggaatgaaaggaaccgcagagtttttcagcaccaagagcttccggtggctagtctgatagccaaaattaaggaggatgccaaaacatgggtcttggcgggcgcgaaacaccttgataggtggcttaccttttaacatgttcgggccaaaggccttgagacggtaaagttttctatttgcgcttgcgcatgtacaattttattcctctattcaatgaaattggtggctcactggttcattaaaaaaaaaagaatctagcctgttcgggaagaagaggattttattcgtgagagagagagagagagagagagagagagggagagagaaggaggaggaggattttcaggcttcgcattgcccaacctctgcttctgttggcccaagaagaatcccaggcgcccatgggctggcagtttaccacggacctacctagcctaccttagctatctaagcgggccgacctagtagctacgtgcctagtgtagattaaagttggcgggccagcaggaagccacgctgcaatggcatcttcccctgtccttcgcgtacgtgaaaacaaacccaggtaagcttagaatcttcttgcccgttggactgggacacccaccaatcccaccatgccccgatattcctccggtctcggttcatgtgatgtcctctcttgtgtgatcacggagcaagcattcttaaacggcaaaagaaaatcaccaacttgctcacgcagtcacgctgcaccgcgcgaagcgacgcccgataggccaagatcgcgagataaaataacaaccaatgatcataaggaaacaagcccgcgatgtgtcgtgtgcagcaatcttggtcatttgcgggatcgagtgcttcacggctaaccaaatattcggccgatgatttaacacattatcagcgtagatgtacgtacgatttgttaattaatctacgagccttgctagggcaggtgttctgccagccaatccagatcgccctcgtatgcacgctcacatgatggcagggcagggttcacatgagctctaacggtcgattaattaatcccggggctcgactataaatacctccctaatcccatgatcaaaacc

SEQ ID NO: 24 - DNA, 99 bp, Oryza sativa
atctcaagcagcctaatcatctccagctgatcaagagctcttaattagctagctagtgattagctgcgcttgtgatcgatcgatctcgggtacgtagca

SEQ ID NO: 25 - DNA, 27 bp, Artificial sequence
  misc_feature (1)..(27): RCc3_Inter_1 amplification primer.
cagcacgttggcgcacacgcccagctt

SEQ ID NO: 26 - DNA, 27 bp, Artificial sequence
  misc_feature (1)..(27): RCc3_Outer_1 amplification primer.
gcacaccgcsgcctcsaggtcgacgag

SEQ ID NO: 27 - DNA, 27 bp, Artificial sequence
  misc_feature (1)..(27): RCc3_Inter_2 amplification primer.
aggttgatgccgagsatgttgsccttg

SEQ ID NO: 28 - DNA, 28 bp, Artificial sequence
  misc_feature (1)..(28): RCc3_Outer_2 amplification primer.
cttgccgcagtrgttgaggakgaggctg

SEQ ID NO: 29 - DNA, 2001 bp, Artificial sequence
  misc_feature (1)..(2001): Codon redesigned GUS coding sequence with processable intron.
atggtgaggcccgttgagaccccgactagggagatcaagaagctggacggcctctgggccttctccctcgaccgtgagaactgcggcatcgaccagcgctggtgggagtccgccctccaggagtctagggccatcgccgtgcccggtttcttcaacgaccagttcgccgacgccgacatccgcaactacgcgggcaacgtctggtatcagcgcgaggtgttcatcccgaagggctgggcgggccagcgcatcgtgctccgcttcgacgccgtgacccactacggcaaggtctgggtgaacaatcaggaggtaagtttctgcttctacctttgatatatatataataattatcattaattagtagtaatataatatttcaaatatttttttcaaaataaaagaatgtagtatatagcaattgcttttctgtagtttataagtgtgtatattttaatttataacttttctaatatatgaccaaaatttgttgatgtgcaggtgatggagcaccagggcggttacaccccgttcgaggccgacgtgacgccgtacgtgatcgccgggaagtccgtccgcatcaccgtctgcgtgaacaatgagctgaactggcagaccatcccgcctggcatggtcatcaccgacgagaacggcaagaagaagcagtcctacttccacgacttcttcaactacgctggcatccaccgctccgtgatgctctacaccactcccaacacctgggtggacgacatcaccgtggtcacccacgtggcccaggactgcaaccacgcctccgtggactggcaagtcgttgccaacggcgacgtcagcgtcgagctgcgcgacgccgaccagcaagtcgttgccaccggccagggcaccagcggcaccctccaagtcgtcaaccctcacctctggcagcctggcgagggctacctctacgagctgtgcgtcaccgccaagagccagactgagtgcgacatctaccctctccgcgtcggcatcaggagcgtcgctgtcaagggcgagcagttcctcatcaaccacaagcctttctacttcactggtttcggccgccacgaggacgctgacctgaggggcaagggtttcgacaacgtcctgatggtccacgaccacgctctgatggactggatcggtgccaacagctacaggaccagtcactacccgtacgctgaggagatgctggactgggctgacgagcacggtatcgtcgtgatcgacgagactgctgcggtcggtttcaacctgtctctgggcattggtttcgaggctgggaacaagccgaaggagctgtactctgaggaagctgtcaacggcgagactcagcaagctcatctccaggcgattaaggagctgattgccagggacaagaaccatccgtctgtcgtgatgtggtctattgcgaatgagccggacaccagaccgcaaggggcgcgtgaatacttcgcgccgctggcggaggcgactcgcaaactggacccaacccgtccaatcacgtgcgtcaatgtcatgttctgcgacgcccatacggatacgatctcggacctgttcgatgttctttgtctcaatcggtactatgggtggtatgttcagagcggggatcttgagacggcggagaaggttcttgagaaggaactcctggcgtggcaagagaagctccatcagccgatcattatcacggagtacggggttgacacacttgcgggccttcacagtatgtacacagatatgtggtcggaggaataccagtgtgcatggttggatatgtaccatcgtgtcttcgaccgggtttcagcggttgtcggcgaacaagtctggaacttcgcagacttcgccacgagccaagggatactgcgggtaggagggaacaagaagggaatcttcacacgggatcggaagcccaagtcagcagccttcctgttgcagaagcgatggacaggaatgaacttcggagaaaagccacagcaaggcggaaagcagtga

SEQ ID NO: 30 - DNA, 1812 bp, Artificial sequence
  misc_feature (1)..(1812): Codong redesigned GUS coding sequence.
atggtgaggcccgttgagaccccgactagggagatcaagaagctggacggcctctgggccttctccctcgaccgtgagaactgcggcatcgaccagcgctggtgggagtccgccctccaggagtctagggccatcgccgtgcccggttccttcaacgaccagttcgccgacgccgacatccgcaactacgcgggcaacgtctggtatcagcgcgaggtgttcatcccgaagggctgggcgggccagcgcatcgtgctccgcttcgacgccgtgacccactacggcaaggtctgggtgaacaatcaggaggtgatggagcaccagggcggttacaccccgttcgaggccgacgtgacgccgtacgtgatcgccgggaagtccgtccgcatcaccgtctgcgtgaacaatgagctgaactggcagaccatcccgcctggcatggtcatcaccgacgagaacggcaagaagaagcagtcctacttccacgacttcttcaactacgctggcatccaccgctccgtgatgctctacaccactcccaacacctgggtggacgacatcaccgtggtcacccacgtggcccaggactgcaaccacgcctccgtggactggcaagtcgttgccaacggcgacgtcagcgtcgagctgcgcgacgccgaccagcaagtcgttgccaccggccagggcaccagcggcaccctccaagtcgtcaaccctcacctctggcagcctggcgagggctacctctacgagctgtgcgtcaccgccaagagccagactgagtgcgacatctaccctctccgcgtcggcatcaggagcgtcgctgtcaagggcgagcagttcctcatcaaccacaagcctttctacttcactggtttcggccgccacgaggacgctgacctgaggggcaagggtttcgacaacgtcctgatggtccacgaccacgctctgatggactggatcggtgccaacagctacaggaccagtcactacccgtacgctgaggagatgctggactgggctgacgagcacggtatcgtcgtgatcgacgagactgctgcggtcggtttcaacctgtctctgggcattggtttcgaggctgggaacaagccgaaggagctgtactctgaggaagctgtcaacggcgagactcagcaagctcatctccaggcgattaaggagctgattgccagggacaagaaccatccgtctgtcgtgatgtggtctattgcgaatgagccggacaccagaccgcaaggggcgcgtgaatacttcgcgccgctggcggaggcgactcgcaaactggacccaacccgtccaatcacgtgcgtcaatgtcatgttctgcgacgcccatacggatacgatctcggacctgttcgatgttctttgtctcaatcggtactatgggtggtatgttcagagcggggatcttgagacggcggagaaggttcttgagaaggaactcctggcgtggcaagagaagctccatcagccgatcattatcacggagtacggggttgacacacttgcgggccttcacagtatgtacacagatatgtggtcggaggaataccagtgtgcatggttggatatgtaccatcgtgtcttcgaccgggtttcagcggttgtcggcgaacaagtctggaacttcgcagacttcgccacgagccaagggatactgcgggtaggagggaacaagaagggaatcttcacacgggatcggaagcccaagtcagcagccttcctgttgcagaagcgatggacaggaatgaacttcggagaaaagccacagcaaggcggaaagcagtga

SEQ ID NO: 31 - DNA, 1812 bp, Escherichia coli
atggtccgtcctgtagaaaccccaacccgtgaaatcaaaaaactcgacggcctgtgggcattcagtctggatcgcgaaaactgtggaattgatcagcgttggtgggaaagcgcgttacaagaaagccgggcaattgctgtgccaggcagttttaacgatcagttcgccgatgcagatattcgtaattatgcgggcaacgtctggtatcagcgcgaagtctttataccgaaaggttgggcaggccagcgtatcgtgctgcgtttcgatgcggtcactcattacggcaaagtgtgggtcaataatcaggaagtgatggagcatcagggcggctatacgccatttgaagccgatgtcacgccgtatgttattgccgggaaaagtgtacgtatcaccgtttgtgtgaacaacgaactgaactggcagactatcccgccgggaatggtgattaccgacgaaaacggcaagaaaaagcagtcttacttccatgatttctttaactatgccggaatccatcgcagcgtaatgctctacaccacgccgaacacctgggtggacgatatcaccgtggtgacgcatgtcgcgcaagactgtaaccacgcgtctgttgactggcaggtggtggccaatggtgatgtcagcgttgaactgcgtgatgcggatcaacaggtggttgcaactggacaaggcactagcgggactttgcaagtggtgaatccgcacctctggcaaccgggtgaaggttatctctatgaactgtgcgtcacagccaaaagccagacagagtgtgatatctacccgcttcgcgtcggcatccggtcagtggcagtgaagggcgaacagttcctgattaaccacaaaccgttctactttactggctttggtcgtcatgaagatgcggacttgcgtggcaaaggattcgataacgtgctgatggtgcacgaccacgcattaatggactggattggggccaactcctaccgtacctcgcattacccttacgctgaagagatgctcgactgggcagatgaacatggcatcgtggtgattgatgaaactgctgctgtcggctttaacctctctttaggcattggtttcgaagcgggcaacaagccgaaagaactgtacagcgaagaggcagtcaacggggaaactcagcaagcgcacttacaggcgattaaagagctgatagcgcgtgacaaaaaccacccaagcgtggtgatgtggagtattgccaacgaaccggatacccgtccgcaaggtgcacgggaatatttcgcgccactggcggaagcaacgcgtaaactcgacccgacgcgtccgatcacctgcgtcaatgtaatgttctgcgacgctcacaccgataccatcagcgatctctttgatgtgctgtgcctgaaccgttattacggatggtatgtccaaagcggcgatttggaaacggcagagaaggtactggaaaaagaacttctggcctggcaggagaaactgcatcagccgattatcatcaccgaatacggcgtggatacgttagccgggctgcactcaatgtacaccgacatgtggagtgaagagtatcagtgtgcatggctggatatgtatcaccgcgtctttgatcgcgtcagcgccgtcgtcggtgaacaggtatggaatttcgccgattttgcgacctcgcaaggcatattgcgcgttggcggtaacaagaaagggatcttcactcgcgaccgcaaaccgaagtcggcggcttttctgctgcaaaaacgctggactggcatgaacttcggtgaaaaaccgcagcagggaggcaaacaatga

SEQ ID NO: 32 - DNA, 2001 bp, Artificial sequence
  misc_feature (1)..(2001): Chimeric coding sequence comprised of the native E. coli GUS coding sequence with a processable intron.
atggtccgtcctgtagaaaccccaacccgtgaaatcaaaaaactcgacggcctgtgggcattcagtctggatcgcgaaaactgtggaattgatcagcgttggtgggaaagcgcgttacaagaaagccgggcaattgctgtgccaggcagttttaacgatcagttcgccgatgcagatattcgtaattatgcgggcaacgtctggtatcagcgcgaagtctttataccgaaaggttgggcaggccagcgtatcgtgctgcgtttcgatgcggtcactcattacggcaaagtgtgggtcaataatcaggaagtgatggagcatcagggcggctatacgccatttgaagccgatgtcacgccgtatgttattgccgggaaaagtgtacgtaagtttctgcttctacctttgatatatatataataattatcattaattagtagtaatataatatttcaaatatttttttcaaaataaaagaatgtagtatatagcaattgcttttctgtagtttataagtgtgtatattttaatttataacttttctaatatatgaccaaaatttgttgatgtgcaggtatcaccgtttgtgtgaacaacgaactgaactggcagactatcccgccgggaatggtgattaccgacgaaaacggcaagaaaaagcagtcttacttccatgatttctttaactatgccggaatccatcgcagcgtaatgctctacaccacgccgaacacctgggtggacgatatcaccgtggtgacgcatgtcgcgcaagactgtaaccacgcgtctgttgactggcaggtggtggccaatggtgatgtcagcgttgaactgcgtgatgcggatcaacaggtggttgcaactggacaaggcactagcgggactttgcaagtggtgaatccgcacctctggcaaccgggtgaaggttatctctatgaactgtgcgtcacagccaaaagccagacagagtgtgatatctacccgcttcgcgtcggcatccggtcagtggcagtgaagggcgaacagttcctgattaaccacaaaccgttctactttactggctttggtcgtcatgaagatgcggacttgcgtggcaaaggattcgataacgtgctgatggtgcacgaccacgcattaatggactggattggggccaactcctaccgtacctcgcattacccttacgctgaagagatgctcgactgggcagatgaacatggcatcgtggtgattgatgaaactgctgctgtcggctttaacctctctttaggcattggtttcgaagcgggcaacaagccgaaagaactgtacagcgaagaggcagtcaacggggaaactcagcaagcgcacttacaggcgattaaagagctgatagcgcgtgacaaaaaccacccaagcgtggtgatgtggagtattgccaacgaaccggatacccgtccgcaaggtgcacgggaatatttcgcgccactggcggaagcaacgcgtaaactcgacccgacgcgtccgatcacctgcgtcaatgtaatgttctgcgacgctcacaccgataccatcagcgatctctttgatgtgctgtgcctgaaccgttattacggatggtatgtccaaagcggcgatttggaaacggcagagaaggtactggaaaaagaacttctggcctggcaggagaaactgcatcagccgattatcatcaccgaatacggcgtggatacgttagccgggctgcactcaatgtacaccgacatgtggagtgaagagtatcagtgtgcatggctggatatgtatcaccgcgtctttgatcgcgtcagcgccgtcgtcggtgaacaggtatggaatttcgccgattttgcgacctcgcaaggcatattgcgcgttggcggtaacaagaaagggatcttcactcgcgaccgcaaaccgaagtcggcggcttttctgctgcaaaaacgctggactggcatgaacttcggtgaaaaaccgcagcagggaggcaaacaatga

SEQ ID NO: 33 - DNA, 435 bp, Setaria italica
ggcgccctttgagaagaagcttttggtctgctgcgcttatcatgttttgtggcttctgtgttgtgattcttgatctgccccttgctatcatttgtattgtactgtcctaataagtggtacttgtgagggtattactgtgtctggttatttacctagaggaggaattattgtctgctatttctggttttgctgtttatgtaatggtgaaccaaagaatgaagctgcaggctactttgagaaggaaggggacctgctgctttctatcttgtcatgcgtgattacttgaacagtcctgatgatctattaatgttctttggtcagtgcaagtgtttggtgtagctccaacaggtagtgtttatgtttggtgaagcagcaatggccgactgtatgtgtttggtgaagctgcaacctgcttgtgctaactgaacatgcaga

SEQ ID NO: 34 - DNA, 2219 bp, Artificial sequence
  misc_feature (1)..(2219): Chimeric transcriptional regulatory expression element group (EXP).
attatggccaattatttatcggcctggtcctggcaggatgagtgtagtagtgtacctaatttggtaggcaatgggtttgagttaggccaataaatgtgcaggtttacatttggttgccatgttagttcataacttcatacacttccatttttgtacgtcggcgatgtttcaaccagaacagattatgtttccttgggactgtaaatttcttcatcgctccatcccaatgaacttgcaagagattcgtgttagcaaccaaaattgctctgtccttcccaaaaagcattgcctctggatcttttccgatcaagatcagaaaccctatatgtattgttcttatgttctgctgtgggtcgttggttcttgtcacccttaaacttctctgtttggtacccagataaatacaaattcggctggtgggtagaaaaaccgcctacgaacactggtttcaccttataagactactgcactgtttctagcaggcttatttttctcttcgttttttatattccaatgtatacatattaatgtttatcgagctatgatcttataaatttgtacatgcttcaatattttctaaaaacttgaataacagtatgtaaaacctaggttgatgtttcaaatgaacttatttaacattttacgttgaaacagtacatcgcgaatggcatattattttgttgcatttattctaaacaccttaaaatggaatttgaaaacgggctctaagtttgagagaagtttaagggtaatagtattctaaacacttcaagtttgagatccaaaataattaatctctcacctatcacctccaatcaagttgtttatcagtttatgccatgtacatgtatcgctggtttgttatttcacctcattttcgctatgtatctactactattgcgctaatctcaaatattagatgacatgtaaactaaaatctttggaaagattaataggatacccgcgggtgctgatatctgtttctaaaaatgttgaatctaactatttgtaaatattgatatatttttcagaaatgttggatttagtcttgtgaaatgttgaaccgatatctctgatatggatttaatgggcttaaagcttccactagccgtgtgcatgggcgaaaaaaaatcttggccaagtgttactccgtcgcggccacacgccacaagtcctcccggccctcgctcgccccttatcccatcgtacccgccacacggcgcgccaccagtggcgccgcggatgcgcctcatctccccggcggccacctcgcgcggtttagatttccctgggcccccctcgcggtaccgtcacatatttttggcgcctcttcttctgcgcccctctcctcccgaaccgcagataccaccgagtcggcagctgaacacaagcaacaagcaagtgatcccggaccgaccgtcttcggtacgcgctcactccgccctctgcctttgttactgccacgtttctctgaatgctctcttgtgtggtgattgctgagagtggtttagctggatctagaattacactctgaaatcgtgttctgcctgtgctgattacttgccgtcctttgtagcagcaaaatatagggacatggtagtacgaaacgaagatagaacctacacagcaatacgagaaatgtgtaatttggtgcttagcggtatttatttaagcacatgttggtgttatagggcacttggattcagaagtttgctgttaatttaggcacaggcttcatactacatgggtcaatagtatagggattcatattataggcgatactataataatttgttcgtctgcagagcttattatttgccaaaattagatattcctattctgtttttgtttgtgtgctgttaaattgttaacgcctgaaggaataaatataaatgacgaaattttgatgtttatctctgctcctttattgtgaccataagtcaagatcagatgcacttgttttaaatattgttgtctgaagaaataagtactgacagtattttgatgcattgatctgcttgtttgttgtaacaaaatttaaaaataaagagtttcctttttgttgctctccttacctcctgatggtatctagtatctaccaactgacactatattgcttctctttacatacgtatcttgctcgatgccttctccctagtgttgaccagtgttactcacatagtctttgctcatttcattgtaatgcagataccaagcgg

SEQ ID NO: 35 - DNA, 2224 bp, Artificial sequence
  misc_feature (1)..(2224): Chimeric transcriptional regulatory expression element group (EXP).
attatggccaattatttatcggcctggtcctggcaggatgagtgtagtagtgtacctaatttggtaggcaatgggtttgagttaggccaataaatgtgcaggtttacatttggttgccatgttagttcataacttcatacacttccatttttgtacgtcggcgatgtttcaaccagaacagattatgtttccttgggactgtaaatttcttcatcgctccatcccaatgaacttgcaagagattcgtgttagcaaccaaaattgctctgtccttcccaaaaagcattgcctctggatcttttccgatcaagatcagaaaccctatatgtattgttcttatgttctgctgtgggtcgttggttcttgtcacccttaaacttctctgtttggtacccagataaatacaaattcggctggtgggtagaaaaaccgcctacgaacactggtttcaccttataagactactgcactgtttctagcaggcttatttttctcttcgttttttatattccaatgtatacatattaatgtttatcgagctatgatcttataaatttgtacatgcttcaatattttctaaaaacttgaataacagtatgtaaaacctaggttgatgtttcaaatgaacttatttaacattttacgttgaaacagtacatcgcgaatggcatattattttgttgcatttattctaaacaccttaaaatggaatttgaaaacgggctctaagtttgagagaagtttaagggtaatagtattctaaacacttcaagtttgagatccaaaataattaatctctcacctatcacctccaatcaagttgtttatcagtttatgccatgtacatgtatcgctggtttgttatttcacctcattttcgctatgtatctactactattgcgctaatctcaaatattagatgacatgtaaactaaaatctttggaaagattaataggatacccgcgggtgctgatatctgtttctaaaaatgttgaatctaactatttgtaaatattgatatatttttcagaaatgttggatttagtcttgtgaaatgttgaaccgatatctctgatatggatttaatgggcttaaagcttccactagccgtgtgcatgggcgaaaaaaaatcttggccaagtgttactccgtcgcggccacacgccacaagtcctcccggccctcgctcgccccttatcccatcgtacccgccacacggcgcgccaccagtggcgccgcggatgcgcctcatctccccggcggccacctcgcgcggtttagatttccctgggcccccctcgcggtaccgtcacatatttttggcgcctcttcttctgcgcccctctcctcccgaaccgcagataccaccgagtcggcagctgaacacaagcaacaagcaagtgatcccggaccggaccgaccgtcttcggtacgcgctcactccgccctctgcctttgttactgccacgtttctctgaatgctctcttgtgtggtgattgctgagagtggtttagctggatctagaattacactctgaaatcgtgttctgcctgtgctgattacttgccgtcctttgtagcagcaaaatatagggacatggtagtacgaaacgaagatagaacctacacagcaatacgagaaatgtgtaatttggtgcttagcggtatttatttaagcacatgttggtgttatagggcacttggattcagaagtttgctgttaatttaggcacaggcttcatactacatgggtcaatagtatagggattcatattataggcgatactataataatttgttcgtctgcagagcttattatttgccaaaattagatattcctattctgtttttgtttgtgtgctgttaaattgttaacgcctgaaggaataaatataaatgacgaaattttgatgtttatctctgctcctttattgtgaccataagtcaagatcagatgcacttgttttaaatattgttgtctgaagaaataagtactgacagtattttgatgcattgatctgcttgtttgttgtaacaaaatttaaaaataaagagtttcctttttgttgctctccttacctcctgatggtatctagtatctaccaactgacactatattgcttctctttacatacgtatcttgctcgatgccttctccctagtgttgaccagtgttactcacatagtctttgctcatttcattgtaatgcagataccaagcgg

SEQ ID NO: 36 - DNA, 2966 bp, Artificial sequence
  misc_feature (1)..(2966): Chimeric transcriptional regulatory expression element group (EXP).
ggtccgattgagacttttcaacaaagggtaatatccggaaacctcctcggattccattgcccagctatctgtcactttattgtgaagatagtggaaaaggaaggtggctcctacaaatgccatcattgcgataaaggaaaggccatcgttgaagatgcctctgccgacagtggtcccaaagatggacccccacccacgaggagcatcgtggaaaaagaagacgttccaaccacgtcttcaaagcaagtggattgatgtgatggtccgattgagacttttcaacaaagggtaatatccggaaacctcctcggattccattgcccagctatctgtcactttattgtgaagatagtggaaaaggaaggtggctcctacaaatgccatcattgcgataaaggaaaggccatcgttgaagatgcctctgccgacagtggtcccaaagatggacccccacccacgaggagcatcgtggaaaaagaagacgttccaaccacgtcttcaaagcaagtggattgatgtgatcggaagctaactagtcacggcgaatacatgacgacatcggcctacaacgcacaacttcttggcataaaagcttcaatttcaatgcccctatctggaagccctaggcgccgcgcaaatgtaaaacattcgcttcgcttggcttgttatccaaaatagagtatggacctccgacagattggcaacccgtgggtaatcgaaaatggctccatctgcccctttgtcgaaggaatcaggaaacggccctcacctcctggcggagtgtagatatgtgaaagaatctaggcgacacttgcagactggacaacatgtgaacaaataagaccaacgttatggcaacaagcctcgacgctactcaagtggtgggaggccaccgcatgttccaacgaagcgccaaagaaagccttgcagactctaatgctattagtcgcctaggatatttggaatgaaaggaaccgcagagtttttcagcaccaagagcttccggtggctagtctgatagccaaaattaaggaggatgccaaaacatgggtcttggcgggcgcgaaacaccttgataggtggcttaccttttaacatgttcgggccaaaggccttgagacggtaaagttttctatttgcgcttgcgcatgtacaattttattcctctattcaatgaaattggtggctcactggttcattaaaaaaaaaagaatctagcctgttcgggaagaagaggattttattcgtgagagagagagagagagagagagagagagggagagagaaggaggaggaggattttcaggcttcgcattgcccaacctctgcttctgttggcccaagaagaatcccaggcgcccatgggctggcagtttaccacggacctacctagcctaccttagctatctaagcgggccgacctagtagctacgtgcctagtgtagattaaagttggcgggccagcaggaagccacgctgcaatggcatcttcccctgtccttcgcgtacgtgaaaacaaacccaggtaagcttagaatcttcttgcccgttggactgggacacccaccaatcccaccatgccccgatattcctccggtctcggttcatgtgatgtcctctcttgtgtgatcacggagcaagcattcttaaacggcaaaagaaaatcaccaacttgctcacgcagtcacgctgcaccgcgcgaagcgacgcccgataggccaagatcgcgagataaaataacaaccaatgatcataaggaaacaagcccgcgatgtgtcgtgtgcagcaatcttggtcatttgcgggatcgagtgcttcacggctaaccaaatattcggccgatgatttaacacattatcagcgtagatgtacgtacgatttgttaattaatctacgagccttgctagggcaggtgttctgccagccaatccagatcgccctcgtatgcacgctcacatgatggcagggcagggttcacatgagctctaacggtcgattaattaatcccggggctcgactataaatacctccctaatcccatgatcaaaaccatctcaagcagcctaatcatctccagctgatcaagagctcttaattagctagctagtgattagctgcgcttgtgatcgatcgatctcgggtacgtagcacggaccggaccgaccgtcttcggtacgcgctcactccgccctctgcctttgttactgccacgtttctctgaatgctctcttgtgtggtgattgctgagagtggtttagctggatctagaattacactctgaaatcgtgttctgcctgtgctgattacttgccgtcctttgtagcagcaaaatatagggacatggtagtacgaaacgaagatagaacctacacagcaatacgagaaatgtgtaatttggtgcttagcggtatttatttaagcacatgttggtgttatagggcacttggattcagaagtttgctgttaatttaggcacaggcttcatactacatgggtcaatagtatagggattcatattataggcgatactataataatttgttcgtctgcagagcttattatttgccaaaattagatattcctattctgtttttgtttgtgtgctgttaaattgttaacgcctgaaggaataaatataaatgacgaaattttgatgtttatctctgctcctttattgtgaccataagtcaagatcagatgcacttgttttaaatattgttgtctgaagaaataagtactgacagtattttgatgcattgatctgcttgtttgttgtaacaaaatttaaaaataaagagtttcctttttgttgctctccttacctcctgatggtatctagtatctaccaactgacactatattgcttctctttacatacgtatcttgctcgatgccttctccctagtgttgaccagtgttactcacatagtctttgctcatttcattgtaatgcagataccaagcgg

SEQ ID NO: 37 - DNA, 2005 bp, Zea mays subsp. Mexicana
gtcgtgcccctctctagagataaagagcattgcatgtctaaagtataaaaaattaccacatatttttttgtcacacttatttgaagtgtagtttatctatctctatacatatatttaaacttcactctacaaataatatagtctataatactaaaataatattagtgttttagaggatcatataaataaactgctagacatggtctaaaggataattgaatattttgacaatctacagttttatctttttagtgtgcatgtgatctctctgttttttttgcaaatagcttgacctatataatacttcatccattttattagtacatccatttaggatttagggttgatggtttctatagactaatttttagtacatccattttattctttttagtctctaaattttttaaaactaaaactctattttagttttttatttaataatttagatataaaatgaaataaaataaattgactacaaataaaacaaataccctttaagaaataaaaaaactaagcaaacatttttcttgtttcgagtagataatgacaggctgttcaacgccgtcgacgagtctaacggacaccaaccagcgaaccagcagcgtcgcgtcgggccaagcgaagcagacggcacggcatctctgtagctgcctctggacccctctcgagagttccgctccaccgttggacttgctccgctgtcggcatccagaaattgcgtggcggagcggcagacgtgaggcggcacggcaggcggcctcttcctcctctcacggcaccggcagctacgggggattcctttcccaccgctccttcgctttcccttcctcgcccgccgtaataaatagacaccccctccacaccctctttccccaacctcgtgttcgttcggagcgcacacacacgcaaccagatctcccccaaatccagccgtcggcacctccgcttcaaggtacgccgctcatcctccccccccccctctctctaccttctctagatcggcgatccggtccatggttagggcccggtagttctacttctgttcatgtttgtgttagagcaaacatgttcatgttcatgtttgtgatgatgtggtctggttgggcggtcgttctagatcggagtaggatactgtttcaagctacctggtggatttattaattttgtatctgtatgtgtgtgccatacatcttcatagttacgagtttaagatgatggatggaaatatcgatctaggataggtatacatgttgatgcgggttttactgatgcatatacagagatgctttttttctcgcttggttgtgatgatatggtctggttgggcggtcgttctagatcggagtagaatactgtttcaaactacctggtggatttattaaaggataaagggtcgttctagatcggagtagaatactgtttcaaactacctggtggatttattaaaggatctgtatgtatgtgcctacatcttcatagttacgagtttaagatgatggatggaaatatcgatctaggataggtatacatgttgatgcgggttttactgatgcatatacagagatgctttttttcgcttggttgtgatgatgtggtctggttgggcggtcgttctagatcggagtagaatactgtttcaaactacctggtggatttattaattttgtatctttatgtgtgtgccatacatcttcatagttacgagtttaagatgatggatggaaatattgatctaggataggtatacatgttgatgtgggttttactgatgcatatacatgatggcatatgcggcatctattcatatgctctaaccttgagtacctatctattataataaacaagtatgttttataattattttgatcttgatatacttggatgatggcatatgcagcagctatatgtggattttttagccctgccttcatacgctatttatttgcttggtactgtttcttttgtccgatgctcaccctgttgttgggtgatacttctgcag

SEQ ID NO: 38 - DNA, 804 bp, Oryza sativa
accgtcttcggtacgcgctcactccgccctctgcctttgttactgccacgtttctctgaatgctctcttgtgtggtgattgctgagagtggtttagctggatctagaattacactctgaaatcgtgttctgcctgtgctgattacttgccgtcctttgtagcagcaaaatatagggacatggtagtacgaaacgaagatagaacctacacagcaatacgagaaatgtgtaatttggtgcttagcggtatttatttaagcacatgttggtgttatagggcacttggattcagaagtttgctgttaatttaggcacaggcttcatactacatgggtcaatagtatagggattcatattataggcgatactataataatttgttcgtctgcagagcttattatttgccaaaattagatattcctattctgtttttgtttgtgtgctgttaaattgttaacgcctgaaggaataaatataaatgacgaaattttgatgtttatctctgctcctttattgtgaccataagtcaagatcagatgcacttgttttaaatattgttgtctgaagaaataagtactgacagtattttgatgcattgatctgcttgtttgttgtaacaaaatttaaaaataaagagtttcctttttgttgctctccttacctcctgatggtatctagtatctaccaactgacactatattgcttctctttacatacgtatcttgctcgatgccttctccctagtgttgaccagtgttactcacatagtctttgctcatttcattgtaatgcagataccaagcgg

SEQ ID NO: 39 - DNA, 253 bp, Agrobacterium tumefaciens
gatcgttcaaacatttggcaataaagtttcttaagattgaatcctgttgccggtcttgcgatgattatcatataatttctgttgaattacgttaagcatgtaataattaacatgtaatgcatgacgttatttatgagatgggtttttatgattagagtcccgcaattatacatttaatacgcgatagaaaacaaaatatagcgcgcaaactaggataaattatcgcgcgcggtgtcatctatgttactagatc

SEQ ID NO: 40 - DNA, 300 bp, Oryza sativa
attaatcgatcctccgatcccttaattaccataccattacaccatgcatcaatatccatatatatataaaccctttcgcacgtacttatactatgttttgtcatacatatatatgtgtcgaacgatcgatctatcactgatatgatatgattgatccatcagcctgatctctgtatcttgttatttgtataccgtcaaataaaagtttcttccacttgtgttaataattagctactctcatctcatgaaccctatatataactagtttaatttgctgtcaattgaacatgatgatcgatg

SEQ ID NO: 41 - DNA, 1446 bp, Artificial sequence
  misc_feature (1)..(1446): Chimeric transcriptional regulatory expression element group (EXP).
ggtccgattgagacttttcaacaaagggtaatatccggaaacctcctcggattccattgcccagctatctgtcactttattgtgaagatagtggaaaaggaaggtggctcctacaaatgccatcattgcgataaaggaaaggccatcgttgaagatgcctctgccgacagtggtcccaaagatggacccccacccacgaggagcatcgtggaaaaagaagacgttccaaccacgtcttcaaagcaagtggattgatgtgatggtccgattgagacttttcaacaaagggtaatatccggaaacctcctcggattccattgcccagctatctgtcactttattgtgaagatagtggaaaaggaaggtggctcctacaaatgccatcattgcgataaaggaaaggccatcgttgaagatgcctctgccgacagtggtcccaaagatggacccccacccacgaggagcatcgtggaaaaagaagacgttccaaccacgtcttcaaagcaagtggattgatgtgatatctccactgacgtaagggatgacgcacaatcccactatccttcgcaagacccttcctctatataaggaagttcatttcatttggagaggacacgctgacaagctgactctagcagatctaccgtcttcggtacgcgctcactccgccctctgcctttgttactgccacgtttctctgaatgctctcttgtgtggtgattgctgagagtggtttagctggatctagaattacactctgaaatcgtgttctgcctgtgctgattacttgccgtcctttgtagcagcaaaatatagggacatggtagtacgaaacgaagatagaacctacacagcaatacgagaaatgtgtaatttggtgcttagcggtatttatttaagcacatgttggtgttatagggcacttggattcagaagtttgctgttaatttaggcacaggcttcatactacatgggtcaatagtatagggattcatattataggcgatactataataatttgttcgtctgcagagcttattatttgccaaaattagatattcctattctgtttttgtttgtgtgctgttaaattgttaacgcctgaaggaataaatataaatgacgaaattttgatgtttatctctgctcctttattgtgaccataagtcaagatcagatgcacttgttttaaatattgttgtctgaagaaataagtactgacagtattttgatgcattgatctgcttgtttgttgtaacaaaatttaaaaataaagagtttcctttttgttgctctccttacctcctgatggtatctagtatctaccaactgacactatattgcttctctttacatacgtatcttgctcgatgccttctccctagtgttgaccagtgttactcacatagtctttgctcatttcattgtaatgcagataccaagcgg

SEQ ID NO: 42 - DNA, 1653 bp, Photinus pyralis
atggaagacgccaaaaacataaagaaaggcccggcgccattctatcctctagaggatggaaccgctggagagcaactgcataaggctatgaagagatacgccctggttcctggaacaattgcttttacagatgcacatatcgaggtgaacatcacgtacgcggaatacttcgaaatgtccgttcggttggcagaagctatgaaacgatatgggctgaatacaaatcacagaatcgtcgtatgcagtgaaaactctcttcaattctttatgccggtgttgggcgcgttatttatcggagttgcagttgcgcccgcgaacgacatttataatgaacgtgaattgctcaacagtatgaacatttcgcagcctaccgtagtgtttgtttccaaaaaggggttgcaaaaaattttgaacgtgcaaaaaaaattaccaataatccagaaaattattatcatggattctaaaacggattaccagggatttcagtcgatgtacacgttcgtcacatctcatctacctcccggttttaatgaatacgattttgtaccagagtcctttgatcgtgacaaaacaattgcactgataatgaattcctctggatctactgggttacctaagggtgtggcccttccgcatagaactgcctgcgtcagattctcgcatgccagagatcctatttttggcaatcaaatcattccggatactgcgattttaagtgttgttccattccatcacggttttggaatgtttactacactcggatatttgatatgtggatttcgagtcgtcttaatgtatagatttgaagaagagctgtttttacgatcccttcaggattacaaaattcaaagtgcgttgctagtaccaaccctattttcattcttcgccaaaagcactctgattgacaaatacgatttatctaatttacacgaaattgcttctgggggcgcacctctttcgaaagaagtcggggaagcggttgcaaaacgcttccatcttccagggatacgacaaggatatgggctcactgagactacatcagctattctgattacacccgagggggatgataaaccgggcgcggtcggtaaagttgttccattttttgaagcgaaggttgtggatctggataccgggaaaacgctgggcgttaatcagagaggcgaattatgtgtcagaggacctatgattatgtccggttatgtaaacaatccggaagcgaccaacgccttgattgacaaggatggatggctacattctggagacatagcttactgggacgaagacgaacacttcttcatagttgaccgcttgaagtctttaattaaatacaaaggatatcaggtggcccccgctgaattggaatcgatattgttacaacaccccaacatcttcgacgcgggcgtggcaggtcttcccgacgatgacgccggtgaacttcccgccgccgttgttgttttggagcacggaaagacgatgacggaaaaagagatcgtggattacgtcgccagtcaagtaacaaccgcgaaaaagttgcgcggaggagttgtgtttgtggacgaagtaccgaaaggtcttaccggaaaactcgacgcaagaaaaatcagagagatcctcataaaggccaagaagggcggaaagtccaaattgtaa

SEQ ID NO: 43 - DNA, 936 bp, Renilla reniformis
atggcttccaaggtgtacgaccccgagcaacgcaaacgcatgatcactgggcctcagtggtgggctcgctgcaagcaaatgaacgtgctggactccttcatcaactactatgattccgagaagcacgccgagaacgccgtgatttttctgcatggtaacgctgcctccagctacctgtggaggcacgtcgtgcctcacatcgagcccgtggctagatgcatcatccctgatctgatcggaatgggtaagtccggcaagagcgggaatggctcatatcgcctcctggatcactacaagtacctcaccgcttggttcgagctgctgaaccttccaaagaaaatcatctttgtgggccacgactggggggcttgtctggcctttcactactcctacgagcaccaagacaagatcaaggccatcgtccatgctgagagtgtcgtggacgtgatcgagtcctgggacgagtggcctgacatcgaggaggatatcgccctgatcaagagcgaagagggcgagaaaatggtgcttgagaataacttcttcgtcgagaccatgctcccaagcaagatcatgcggaaactggagcctgaggagttcgctgcctacctggagccattcaaggagaagggcgaggttagacggcctaccctctcctggcctcgcgagatccctctcgttaagggaggcaagcccgacgtcgtccagattgtccgcaactacaacgcctaccttcgggccagcgacgatctgcctaagatgttcatcgagtccgaccctgggttcttttccaacgctattgtcgagggagctaagaagttccctaacaccgagttcgtgaaggtgaagggcctccacttcagccaggaggacgctccagatgaaatgggtaagtacatcaagagcttcgtggagcgcgtgctgaagaacgagcagtaa

SEQ ID NO: 44 - DNA, 675 bp, Artificial sequence
  misc_feature (1)..(675): Chimeric transcriptional regulatory expression element group (EXP).
ggtccgatgtgagacttttcaacaaagggtaatatccggaaacctcctcggattccattgcccagctatctgtcactttattgtgaagatagtggaaaaggaaggtggctcctacaaatgccatcattgcgataaaggaaaggccatcgttgaagatgcctctgccgacagtggtcccaaagatggacccccacccacgaggagcatcgtggaaaaagaagacgttccaaccacgtcttcaaagcaagtggattgatgtgatggtccgatgtgagacttttcaacaaagggtaatatccggaaacctcctcggattccattgcccagctatctgtcactttattgtgaagatagtggaaaaggaaggtggctcctacaaatgccatcattgcgataaaggaaaggccatcgttgaagatgcctctgccgacagtggtcccaaagatggacccccacccacgaggagcatcgtggaaaaagaagacgttccaaccacgtcttcaaagcaagtggattgatgtgatatctccactgacgtaagggatgacgcacaatcccactatccttcgcaagacccttcctctatataaggaagttcatttcatttggagaggaaccatcttccacacactcaagccacactattggagaacacacagggacaacacaccataa